European Patent Specification EP 3 345 613 B1, published May 10, 2023. Title: PHARMACEUTICAL COMPOSITION CONTAINING, AS ACTIVE INGREDIENT, FUSION PROTEIN IN WHICH TUMOR-PENETRATING PEPTIDE AND ANTI-ANGIOGENESIS AGENT ARE FUSED, FOR PREVENTING AND TREATING CANCER OR ANGIOGENESIS-RELATED DISEASES. Applicant: IL DONG PHARMACEUTICAL CO., LTD. Application 16842324.2. The sequence listing filed with the application follows.

SEQUENCE LISTING (13 sequences)

SEQ ID NO: 1 - protein, 22 aa, Artificial Sequence
  TPP#1
HTPGNSNKWKHLQENKKGRNRR

SEQ ID NO: 2 - protein, 22 aa, Artificial Sequence
  TPP#2
HTPGNSNKWKHLQENKKGRPRR

SEQ ID NO: 3 - protein, 22 aa, Artificial Sequence
  TPP#3
REAPGAPRSPEPQDQKKPRNRR

SEQ ID NO: 4 - protein, 22 aa, Artificial Sequence
  TPP#4
REAPGAPRSPEPQDQKKPRPRR

SEQ ID NO: 5 - protein, 18 aa, Artificial Sequence
  TPP#5
HTPGNSNQFVLTSTRPPR

SEQ ID NO: 6 - protein, 11 aa, Artificial Sequence
  TPP#6
HTPGIATRTPR

SEQ ID NO: 7 - protein, 14 aa, Artificial Sequence
  TPP#7
HTPGNSKPTRTPRR

SEQ ID NO: 8 - protein, 15 aa, Artificial Sequence
  Linker
GGGGSGGGGSGGGGS

SEQ ID NO: 9 - protein, 490 aa, Artificial Sequence
  Avastin-HC-A22p
EVQLVESGGGLVQPGGSLRLSCAASGYTFTNYGMNWVRQAPGKGLEWVGWINTYTGEPTYAADFKRRFTFSLDTSKSTAYLQMNSLRAEDTAVYYCAKYPHYYGSSHWYFDVWGQGTLVTVSSASTKGPSVFPLAPSSKSTSGGTAALGCLVKDYFPEPVTVSWNSGALTSGVHTFPAVLQSSGLYSLSSVVTVPSSSLGTQTYICNVNHKPSNTKVDKKVEPKSCDKTHTCPPCPAPELLGGPSVFLFPPKPKDTLMISRTPEVTCVVVDVSHEDPEVKFNWYVDGVEVHNAKTKPREEQYNSTYRVVSVLTVLHQDWLNGKEYKCKVSNKALPAPIEKTISKAKGQPREPQVYTLPPSREEMTKNQVSLTCLVKGFYPSDIAVEWESNGQPENNYKTTPPVLDSDGSFFLYSKLTVDKSRWQQGNVFSCSVMHEALHNHYTQKSLSLSPGKGGGGSGGGGSGGGGSHTPGNSNKWKHLQENKKGRPRR

SEQ ID NO: 10 - protein, 482 aa, Artificial Sequence
  Avastin-HC-TPP11
EVQLVESGGGLVQPGGSLRLSCAASGYTFTNYGMNWVRQAPGKGLEWVGWINTYTGEPTYAADFKRRFTFSLDTSKSTAYLQMNSLRAEDTAVYYCAKYPHYYGSSHWYFDVWGQGTLVTVSSASTKGPSVFPLAPSSKSTSGGTAALGCLVKDYFPEPVTVSWNSGALTSGVHTFPAVLQSSGLYSLSSVVTVPSSSLGTQTYICNVNHKPSNTKVDKKVEPKSCDKTHTCPPCPAPELLGGPSVFLFPPKPKDTLMISRTPEVTCVVVDVSHEDPEVKFNWYVDGVEVHNAKTKPREEQYNSTYRVVSVLTVLHQDWLNGKEYKCKVSNKALPAPIEKTISKAKGQPREPQVYTLPPSREEMTKNQVSLTCLVKGFYPSDIAVEWESNGQPENNYKTTPPVLDSDGSFFLYSKLTVDKSRWQQGNVFSCSVMHEALHNHYTQKSLSLSPGKGGGGSGGGGSGGGGSHTPGNSKPTRTPRR

SEQ ID NO: 11 - protein, 214 aa, Artificial Sequence
  Avastin-LC
DIQMTQSPSSLSASVGDRVTITCSASQDISNYLNWYQQKPGKAPKVLIYFTSSLHSGVPSRFSGSGSGTDFTLTISSLQPEDFATYYCQQYSTVPWTFGQGTKVEIKRTVAAPSVFIFPPSDEQLKSGTASVVCLLNNFYPREAKVQWKVDNALQSGNSQESVTEQDSKDSTYSLSSTLTLSKADYEKHKVYACEVTHQGLSSPVTKSFNRGEC

SEQ ID NO: 12 - protein, 490 aa, Artificial Sequence
  Avastin(V)-HC-A22p
EVQLVESGGGLVQPGGSLRLSCAASGYTFTNYGMNWVRQAPGKGLEWVGWINTYTGEPTYAADFKRRFTFSLDTSKSTAYLQMNSLRAEDTAVYYCAKYPHYYGSSHWYFDVWGQGTLVTVSSASTKGPSVFPLAPSSKSTSGGTAALGCLVKDYFPEPVTVSWNSGALTSGVHTFPAVLQSSGLYSLSSVVTVPSSSLGTQTYICNVNHKPSNTKVDKKVEPKSCDKTHTCPPCPAPELLGGPSVFLFPPKPKDTLMISRTPEVTCVVVDVSHEDPEVKFNWYVDGVEVHNAKTKPREEQYNSTYRVVSVLTVLHQDWLNGKEYKCKVSNKALPAPIEKTISKAKGQPREPQVYTLPPSRDELTKNQVSLTCLVKGFYPSDIAVEWESNGQPENNYKTTPPVLDSDGSFFLYSKLTVDKSRWQQGNVFSCSVMHEALHNHYTQKSLSLSPGKGGGGSGGGGSGGGGSHTPGNSNKWKHLQENKKGRPRR

SEQ ID NO: 13 - protein, 453 aa, Artificial Sequence
  Avastin-HC
EVQLVESGGGLVQPGGSLRLSCAASGYTFTNYGMNWVRQAPGKGLEWVGWINTYTGEPTYAADFKRRFTFSLDTSKSTAYLQMNSLRAEDTAVYYCAKYPHYYGSSHWYFDVWGQGTLVTVSSASTKGPSVFPLAPSSKSTSGGTAALGCLVKDYFPEPVTVSWNSGALTSGVHTFPAVLQSSGLYSLSSVVTVPSSSLGTQTYICNVNHKPSNTKVDKKVEPKSCDKTHTCPPCPAPELLGGPSVFLFPPKPKDTLMISRTPEVTCVVVDVSHEDPEVKFNWYVDGVEVHNAKTKPREEQYNSTYRVVSVLTVLHQDWLNGKEYKCKVSNKALPAPIEKTISKAKGQPREPQVYTLPPSREEMTKNQVSLTCLVKGFYPSDIAVEWESNGQPENNYKTTPPVLDSDGSFFLYSKLTVDKSRWQQGNVFSCSVMHEALHNHYTQKSLSLSPGK